European Patent Application EP 4 197 545 A1, published June 21, 2023. Title: Pharmaceutical composition comprising cell expressing chimeric receptor. Applicant: CHUGAI SEIYAKU KABUSHIKI KAISHA. The sequence listing filed with the application follows.

SEQUENCE LISTING (140 sequences)

SEQ ID NO: 1 - protein, 115 aa, Artificial Sequence
  an artificially synthesized sequence
QVQLVQSGAEVKKPGASVKVSCKASGYTFTDYEMHWIRQPPGQGLEWIGAIDPKTGDTAYSQKFKGRVTLTADKSTSTAYMELSSLTSEDTAVYYCTRFYSYTYWGQGTLVTVSS

SEQ ID NO: 2 - protein, 112 aa, Artificial Sequence
  an artificially synthesized sequence
DIVMTQSPLSLPVTPGEPASISCRSSQSLVHSNRNTYLHWYQQKPGQAPRLLIYKVSNRFSGVPDRFSGSGSGTDFTLKISRVEAEDVGVYYCSQNTHVPPTFGQGTKLEIK

SEQ ID NO: 3 - protein, 328 aa, Artificial Sequence
  an artificially synthesized sequence
ASTKGPSVFPLAPSSKSTSGGTAALGCLVKDYFPEPVTVSWNSGALTSGVHTFPAVLQSSGLYSLSSVVTVPSSSLGTQTYICNVNHKPSNTKVDKKVEPKSCDKTHTCPPCPAPELRGGPKVFLFPPKPKDTLMISRTPEVTCVVVDVSHEDPEVKFNWYVDGVEVHNAKTKPREEQYASTYRVVSVLTVLHQDWLNGKEYKCKVSNKALPAPIEKTISKAKGQPREPQVYTLPPSRDELTKNQVSLTCLVKGFYPSDIAVEWESNGQPENNYKTTPPYLDSDGSFFLYSKLTVDKSRWQQGNVFSCSVMHEALHNHYTQESLSLSP

SEQ ID NO: 4 - protein, 107 aa, Artificial Sequence [sequence omitted]

SEQ ID NO: 5 - protein, 121 aa, Artificial Sequence [sequence omitted]

SEQ ID NO: 6 - protein, 109 aa, Artificial Sequence [sequence omitted]

SEQ ID NO: 7 - protein, 328 aa, Artificial Sequence
  an artificially synthesized sequence
ASTKGPSVFPLAPSSKSTSGGTAALGCLVKDYFPEPVTVSWNSGALTSGVHTFPAVLQSSGLYSLSSVVTVPSSSLGTQTYICNVNHKPSNTKVDKKVEPKSCDKTHTCPPCPAPELRGGPKVFLFPPKPKDTLMISRTPEVTCVVVDVSHEDPEVKFNWYVDGVEVHNAKTKPREEQYASTYRVVSVLTVLHQDWLNGKEYKCKVSNKALPAPIEKTISKAKGQPREPQVYTLPPSRKEMTKNQVSLTCLVKGFYPSDIAVEWESNGQPENNYKTTPPYLDSDGSFFLYSKLTVDKSRWQQGNVFSCSVMHEALHNHYTQKSLSLSP

SEQ ID NO: 8 - protein, 107 aa, Artificial Sequence [sequence omitted]

SEQ ID NO: 9 - protein, 116 aa, Artificial Sequence
  an artificially synthesized sequence
QSVEESGGRLVTPGTPLTLTCTVSGFSLSSYAMSWVRQAPGKGLEWIGIINIRGSTYYASWAKGRFTISKTSTTVDLKITSPTTADTATYFCARGYTAYSGAVSIWGPGTLVTVSS

SEQ ID NO: 10 - protein, 110 aa, Artificial Sequence
  an artificially synthesized sequence
DVVMTQTPASVSEPVGGTVTIKCQASQNIYSNLAWYQQKPGQPPKLLIYAASNLASGVSSRFKGSGSGTQFTLTISDLECADSATYYCQCSDYGSSYVGAFGGGTEVVVK

SEQ ID NO: 11 - protein, 328 aa, Artificial Sequence
  an artificially synthesized sequence
ASTKGPSVFPLAPSSKSTSGGTAALGCLVKDYFPEPVTVSWNSGALTSGVHTFPAVLQSSGLYSLSSVVTVPSSSLGTQTYICNVNHKPSNTKVDKKVEPKSCDKTHTCPPCPAPELRGGPKVFLFPPKPKDTLMISRTPEVTCVVVDVSHEDPEVKFNWYVDGVEVHNAKTKPREEQYASTYRVVSVLTVLHQDWLNGKEYKCKVSNKALPAPIEKTISKAKGQPREPQVYTLPPSREEMTKNQVSLTCLVKGFYPSDIAVEWESNGQPENNYKTTPPYLDSDGSFFLYSKLTVDKSRWQQGNVFSCSVMHEALHNHYTQESLSLSP

SEQ ID NO: 12 - protein, 107 aa, Artificial Sequence
  an artificially synthesized sequence
RTVAAPSVFIFPPSDEQLKSGTASVVCLLNNFYPREAKVQWKVDNALQSGNSQESVTEQDSKDCTYSLSSTLTLSKADYEKHKVYACEVTHQGLSSPVTKSFNRGEC

SEQ ID NO: 13 - protein, 119 aa, Artificial Sequence
  an artificially synthesized sequence
QSVEESGGRLVTPGGTLTFTCTVSGFSLSSYAMGWVRQAPGEGLEYIGTIDTGGSAYYATWAKGRFTISKTSSTTVGLIMTSLTAADTATYFCARVADYNIGLRRLDLWGQGTLVTVSS

SEQ ID NO: 14 - protein, 111 aa, Artificial Sequence
  an artificially synthesized sequence
ADVVMTQTPASVSEPVGGTVTIKCQASQYIYSNLAWYQQKPGQRPKLLIYTTSNLESGVPSRFRGSGSGTEFTLTISDLECADAATYYCQSAYYSSSYVFPFGGGTEVVVK

SEQ ID NO: 15 - protein, 119 aa, Artificial Sequence [sequence omitted]

SEQ ID NO: 16 - protein, 107 aa, Artificial Sequence [sequence omitted]

SEQ ID NO: 17 - protein, 107 aa, Artificial Sequence [sequence omitted]

SEQ ID NO: 18 - protein, 116 aa, Artificial Sequence
  an artificially synthesized sequence
QVQLQQSGPQLVRPGASVKISCKASGYSFTSYWMHWVNQRPGQGLEWIGMIDPSYSETRLNQKFKDKATLTVDKSSSTAYMQLSSPTSEDSAVYYCALYGNYFDYWGQGTTLTVSS

SEQ ID NO: 19 - protein, 107 aa, Artificial Sequence
  an artificially synthesized sequence
DIQMTQSSSSFSVSLGDRVTITCKASEDIYNRLAWYQQKPGNAPRLLISGATSLETGVPSRFSGSGSGKDYTLSITSLQTEDVATYYCQQYWSTPYTFGGGTKLEVK

SEQ ID NO: 20 - protein, 120 aa, Artificial Sequence
  an artificially synthesized sequence
QVQLVQSGAEVKKPGASVKVSCKASGYTFTSYYIHWVRQAPGQGLEWIGCIYPGNVNTNYNEKFKDRATLTVDTSISTAYMELSRLRSDDTAVYFCTRSHYGLDWNFDVWGQGTTVTVSS

SEQ ID NO: 21 - protein, 107 aa, Artificial Sequence
  an artificially synthesized sequence
DIQMTQSPSSLSASVGDRVTITCHASQNTYVWLNWYQQKPGKAPKLLIYKASNLHTGVPSRFSGSGSGTDFTLTISSLQPEDFATYYCQQGQTYPYTFGGGTKVEIK

SEQ ID NO: 22 - protein, 328 aa, Artificial Sequence; identical to SEQ ID NO: 7
  an artificially synthesized sequence

SEQ ID NO: 23 - protein, 107 aa, Artificial Sequence [sequence omitted]

SEQ ID NO: 24 - protein, 449 aa, Artificial Sequence
  an artificially synthesized sequence
LQDPCSNCPAGTFCDNNRNQICSPCPPNSFSSAGGQRTCDICRQCKGVFRTRKECSSTSNAECDCTPGFHCLGAGCSMCEQDCKQGQELTKKGCKDCCFGTFNDQKRGICRPWTNCSLDGKSVLVNGTKERDVVCGPSPADLSPGASSVTPPAPAREPGHSPQAAAFVPVFLPAKPTTTPAPRPPTPAPTIASQPLSLRPEACRPAAGGAVHTRGLDFACDIYIWAPLAGTCGVLLLSLVITLYCNHRNRSKRSRLLHSDYMNMTPRRPGPTRKHYQPYAPPRDFAAYRSRFSVVKRGRKKLLYIFKQPFMRPVQTTQEEDGCSCRFPEEEEGGCELRVKFSRSADAPAYQQGQNQLYNELNLGRREEYDVLDKRRGRDPEMGGKPRRKNPQEGLYNELQKDKMAEAYSEIGMKGERRRGKGHDGLYQGLSTATKDTYDALHMQALPPR

SEQ ID NO: 25 - protein, 350 aa, Artificial Sequence
  an artificially synthesized sequence
LQDPCSNCPAGTFCDNNRNQICSPCPPNSFSSAGGQRTCDICRQCKGVFRTRKECSSTSNAECDAAAFVPVFLPAKPTTTPAPRPPTPAPTIASQPLSLRPEACRPAAGGAVHTRGLDFACDIYIWAPLAGTCGVLLLSLVITLYCNHRNRSKRSRLLHSDYMNMTPRRPGPTRKHYQPYAPPRDFAAYRSRFSVVKRGRKKLLYIFKQPFMRPVQTTQEEDGCSCRFPEEEEGGCELRVKFSRSADAPAYQQGQNQLYNELNLGRREEYDVLDKRRGRDPEMGGKPRRKNPQEGLYNELQKDKMAEAYSEIGMKGERRRGKGHDGLYQGLSTATKDTYDALHMQALPPR

SEQ ID NO: 26 - protein, 449 aa, Artificial Sequence
  an artificially synthesized sequence
LQDPCSNCPAGTFCDNNRNQICSPCPPNSFSSAGGQRTCDRCRQCKGRFRTRKECSSTSNAECDCTPGFHCLGAGCSMCEQDCKQGQELTKKGCKDCCFGTFNDQKRGICRPWTNCSLDGKSVLVNGTKERDVVCGPSPADLSPGASSVTPPAPAREPGHSPQAAAFVPVFLPAKPTTTPAPRPPTPAPTIASQPLSLRPEACRPAAGGAVHTRGLDFACDIYIWAPLAGTCGVLLLSLVITLYCNHRNRSKRSRLLHSDYMNMTPRRPGPTRKHYQPYAPPRDFAAYRSRFSVVKRGRKKLLYIFKQPFMRPVQTTQEEDGCSCRFPEEEEGGCELRVKFSRSADAPAYQQGQNQLYNELNLGRREEYDVLDKRRGRDPEMGGKPRRKNPQEGLYNELQKDKMAEAYSEIGMKGERRRGKGHDGLYQGLSTATKDTYDALHMQALPPR

SEQ ID NO: 27 - protein, 449 aa, Artificial Sequence
  an artificially synthesized sequence
LQDPCSNCPAGTFCDNNRNQICSPCPPNSFSSAGGQRTCDICRQCKGEFRTRKECSSTSNAECDCTPGFHCLGAGCSMCEQDCKQGQELTKKGCKDCCFGTFNDQKRGICRPWTNCSLDGKSVLVNGTKERDVVCGPSPADLSPGASSVTPPAPAREPGHSPQAAAFVPVFLPAKPTTTPAPRPPTPAPTIASQPLSLRPEACRPAAGGAVHTRGLDFACDIYIWAPLAGTCGVLLLSLVITLYCNHRNRSKRSRLLHSDYMNMTPRRPGPTRKHYQPYAPPRDFAAYRSRFSVVKRGRKKLLYIFKQPFMRPVQTTQEEDGCSCRFPEEEEGGCELRVKFSRSADAPAYQQGQNQLYNELNLGRREEYDVLDKRRGRDPEMGGKPRRKNPQEGLYNELQKDKMAEAYSEIGMKGERRRGKGHDGLYQGLSTATKDTYDALHMQALPPR

SEQ ID NO: 28 - protein, 449 aa, Artificial Sequence
  an artificially synthesized sequence
LQDPCSNCPAGTFCDNNRNQICSPCPPNSFSSAGGQRTCDICRQCKGQFRTRKECSSTSNAECDCTPGFHCLGAGCSMCEQDCKQGQELTKKGCKDCCFGTFNDQKRGICRPWTNCSLDGKSVLVNGTKERDVVCGPSPADLSPGASSVTPPAPAREPGHSPQAAAFVPVFLPAKPTTTPAPRPPTPAPTIASQPLSLRPEACRPAAGGAVHTRGLDFACDIYIWAPLAGTCGVLLLSLVITLYCNHRNRSKRSRLLHSDYMNMTPRRPGPTRKHYQPYAPPRDFAAYRSRFSVVKRGRKKLLYIFKQPFMRPVQTTQEEDGCSCRFPEEEEGGCELRVKFSRSADAPAYQQGQNQLYNELNLGRREEYDVLDKRRGRDPEMGGKPRRKNPQEGLYNELQKDKMAEAYSEIGMKGERRRGKGHDGLYQGLSTATKDTYDALHMQALPPR

SEQ ID NO: 29 - protein, 449 aa, Artificial Sequence
  an artificially synthesized sequence
LQDPCSNCPAGTFCDNNRNQICSPCPPNSFSSAGGQRTCDECRQCKGQFRTRKECSSTSNAECDCTPGFHCLGAGCSMCEQDCKQGQELTKKGCKDCCFGTFNDQKRGICRPWTNCSLDGKSVLVNGTKERDVVCGPSPADLSPGASSVTPPAPAREPGHSPQAAAFVPVFLPAKPTTTPAPRPPTPAPTIASQPLSLRPEACRPAAGGAVHTRGLDFACDIYIWAPLAGTCGVLLLSLVITLYCNHRNRSKRSRLLHSDYMNMTPRRPGPTRKHYQPYAPPRDFAAYRSRFSVVKRGRKKLLYIFKQPFMRPVQTTQEEDGCSCRFPEEEEGGCELRVKFSRSADAPAYQQGQNQLYNELNLGRREEYDVLDKRRGRDPEMGGKPRRKNPQEGLYNELQKDKMAEAYSEIGMKGERRRGKGHDGLYQGLSTATKDTYDALHMQALPPR

SEQ ID NO: 30 - protein, 449 aa, Artificial Sequence
  an artificially synthesized sequence
LQDPCSNCPAGTFCDNNRNQICSPCPPNSFSSAGGQRTCDQCRQCKGEFRTRKECSSTSNAECDCTPGFHCLGAGCSMCEQDCKQGQELTKKGCKDCCFGTFNDQKRGICRPWTNCSLDGKSVLVNGTKERDVVCGPSPADLSPGASSVTPPAPAREPGHSPQAAAFVPVFLPAKPTTTPAPRPPTPAPTIASQPLSLRPEACRPAAGGAVHTRGLDFACDIYIWAPLAGTCGVLLLSLVITLYCNHRNRSKRSRLLHSDYMNMTPRRPGPTRKHYQPYAPPRDFAAYRSRFSVVKRGRKKLLYIFKQPFMRPVQTTQEEDGCSCRFPEEEEGGCELRVKFSRSADAPAYQQGQNQLYNELNLGRREEYDVLDKRRGRDPEMGGKPRRKNPQEGLYNELQKDKMAEAYSEIGMKGERRRGKGHDGLYQGLSTATKDTYDALHMQALPPR

SEQ ID NO: 31 - protein, 449 aa, Artificial Sequence
  an artificially synthesized sequence
LQDPCSNCPAGTFCDNNRNQICSPCPPNSFSSAGGQRTCDQCRQCKGQFRTRKECSSTSNAECDCTPGFHCLGAGCSMCEQDCKQGQELTKKGCKDCCFGTFNDQKRGICRPWTNCSLDGKSVLVNGTKERDVVCGPSPADLSPGASSVTPPAPAREPGHSPQAAAFVPVFLPAKPTTTPAPRPPTPAPTIASQPLSLRPEACRPAAGGAVHTRGLDFACDIYIWAPLAGTCGVLLLSLVITLYCNHRNRSKRSRLLHSDYMNMTPRRPGPTRKHYQPYAPPRDFAAYRSRFSVVKRGRKKLLYIFKQPFMRPVQTTQEEDGCSCRFPEEEEGGCELRVKFSRSADAPAYQQGQNQLYNELNLGRREEYDVLDKRRGRDPEMGGKPRRKNPQEGLYNELQKDKMAEAYSEIGMKGERRRGKGHDGLYQGLSTATKDTYDALHMQALPPR

SEQ ID NO: 32 - protein, 449 aa, Artificial Sequence
  an artificially synthesized sequence
LQDPCSNCPAGTFCDNNRNQICSPCPPNSFSSAGGQRTCDICRQCKGVFRTRKECSSTSNAECDCTPGFHCLGAGCSDCEQDCKQGQELTKKGCKDCCFGTFNDQKRGICRPWTNCSLDGKSVLVNGTKERDVVCGPSPADLSPGASSVTPPAPAREPGHSPQAAAFVPVFLPAKPTTTPAPRPPTPAPTIASQPLSLRPEACRPAAGGAVHTRGLDFACDIYIWAPLAGTCGVLLLSLVITLYCNHRNRSKRSRLLHSDYMNMTPRRPGPTRKHYQPYAPPRDFAAYRSRFSVVKRGRKKLLYIFKQPFMRPVQTTQEEDGCSCRFPEEEEGGCELRVKFSRSADAPAYQQGQNQLYNELNLGRREEYDVLDKRRGRDPEMGGKPRRKNPQEGLYNELQKDKMAEAYSEIGMKGERRRGKGHDGLYQGLSTATKDTYDALHMQALPPR

SEQ ID NO: 33 - protein, 362 aa, Artificial Sequence
  an artificially synthesized sequence
LQDPCSNCPAGTFCDNNRNQICSPCPPNSFSSAGGQRTCDICRQCKGVFRTRKECSSTSNAECDCTPGFHCLGAGCSMCEQDCKQGQELTKKGCKDCCFGTFNDQKRGICRPWTNCSLDGKSVLVNGTKERDVVCGPSPADLSPGASSVTPPAPAREPGHSPQAAAFVPVFLPAKPTTTPAPRPPTPAPTIASQPLSLRPEACRPAAGGAVHTRGLDFACDIYIWAPLAGTCGVLLLSLVITLYCNHRNRRVKFSRSADAPAYQQGQNQLYNELNLGRREEYDVLDKRRGRDPEMGGKPRRKNPQEGLYNELQKDKMAEAYSEIGMKGERRRGKGHDGLYQGLSTATKDTYDALHMQALPPR

SEQ ID NO: 34 - protein, 420 aa, Artificial Sequence
  an artificially synthesized sequence
NKILVKQSPMLVAYDNAVNLSCKYSYNLFSREFRASLHKGLDSAVEVCVVYGNYSQQLQVYSKTGFNCDGKLGNESVTFYLQNLYVNQTDIYFCKIEVMYPPPYLDNEKSNGTIIHVKGKHLCPSPLFPGPSKPAAAFVPVFLPAKPTTTPAPRPPTPAPTIASQPLSLRPEACRPAAGGAVHTRGLDFACDIYIWAPLAGTCGVLLLSLVITLYCNHRNRSKRSRLLHSDYMNMTPRRPGPTRKHYQPYAPPRDFAAYRSRFSVVKRGRKKLLYIFKQPFMRPVQTTQEEDGCSCRFPEEEEGGCELRVKFSRSADAPAYQQGQNQLYNELNLGRREEYDVLDKRRGRDPEMGGKPRRKNPQEGLYNELQKDKMAEAYSEIGMKGERRRGKGHDGLYQGLSTATKDTYDALHMQALPPR

SEQ ID NO: 35 - protein, 361 aa, Artificial Sequence
  an artificially synthesized sequence
NKILVKQSPMLVAYDNAVNLSCKYSYNLFSREFRASLHKGLDSAVEVCVVYGNYSQQLQVYSKTGFNCDGKLGNESVTFYLQNLYVNQTDIYFCKIEVMYPPPYLDNEKSNGTIIHVKGKHLCPSPLFPGPSKPFWVLVVVGGVLACYSLLVTVAFIIFWVRSKRSRLLHSDYMNMTPRRPGPTRKHYQPYAPPRDFAAYRSRFSVVKRGRKKLLYIFKQPFMRPVQTTQEEDGCSCRFPEEEEGGCELRVKFSRSADAPAYQQGQNQLYNELNLGRREEYDVLDKRRGRDPEMGGKPRRKNPQEGLYNELQKDKMAEAYSEIGMKGERRRGKGHDGLYQGLSTATKDTYDALHMQALPPR

SEQ ID NO: 36 - protein, 163 aa, Artificial Sequence
  an artificially synthesized sequence
LQDPCSNCPAGTFCDNNRNQICSPCPPNSFSSAGGQRTCDICRQCKGVFRTRKECSSTSNAECDCTPGFHCLGAGCSMCEQDCKQGQELTKKGCKDCCFGTFNDQKRGICRPWTNCSLDGKSVLVNGTKERDVVCGPSPADLSPGASSVTPPAPAREPGHSPQ

SEQ ID NO: 37 - protein, 7 aa, Artificial Sequence
  an artificially synthesized sequence
DIEGRMD

SEQ ID NO: 38 - protein, 229 aa, Artificial Sequence
  an artificially synthesized sequence
PKSCDKTHTCPPCPAPELLGGPSVFLFPPKPKDTLMISRTPEVTCVVVDVSHEDPEVKFNWYVDGVEVHNAKTKPREEQYNSTYRVVSVLTVLHQDWLNGKEYKCKVSNKALPAPIEKTISKAKGQPREPQVYTLPPSREEMTKNQVSLTCLVKGFYPSDIAVEWESNGQPENNYKTTPPVLDSDGSFFLYSKLTVDKSRWQQGNVFSCSVMHEALHNHYTQKSLSLSP

SEQ ID NO: 39 - protein, 20 aa, Artificial Sequence
  an artificially synthesized sequence
GGGGSGLNDIFEAQKIEWHE

SEQ ID NO: 40 - protein, 163 aa, Artificial Sequence
  an artificially synthesized sequence
LQDPCSNCPAGTFCDNNRNQICSPAPPNSFSSAGGQRTCDICRQCKGVFRTRKECSSTSNAECDCTPGFHCLGAGCSMCEQDCKQGQELTKKGCKDCCFGTFNDQKRGICRPWTNCSLDGKSVLVNGTKERDVVCGPSPADLSPGASSVTPPAPAREPGHSPQ

SEQ ID NO: 41 - protein, 163 aa, Artificial Sequence
  an artificially synthesized sequence
LQDPCSNCPAGTFCDNNRNQICSPCAPNSFSSAGGQRTCDICRQCKGVFRTRKECSSTSNAECDCTPGFHCLGAGCSMCEQDCKQGQELTKKGCKDCCFGTFNDQKRGICRPWTNCSLDGKSVLVNGTKERDVVCGPSPADLSPGASSVTPPAPAREPGHSPQ

SEQ ID NO: 42 - protein, 163 aa, Artificial Sequence
  an artificially synthesized sequence
LQDPCSNCPAGTFCDNNRNQICSPCPANSFSSAGGQRTCDICRQCKGVFRTRKECSSTSNAECDCTPGFHCLGAGCSMCEQDCKQGQELTKKGCKDCCFGTFNDQKRGICRPWTNCSLDGKSVLVNGTKERDVVCGPSPADLSPGASSVTPPAPAREPGHSPQ

SEQ ID NO: 43 - protein, 163 aa, Artificial Sequence
  an artificially synthesized sequence
LQDPCSNCPAGTFCDNNRNQICSPCPPASFSSAGGQRTCDICRQCKGVFRTRKECSSTSNAECDCTPGFHCLGAGCSMCEQDCKQGQELTKKGCKDCCFGTFNDQKRGICRPWTNCSLDGKSVLVNGTKERDVVCGPSPADLSPGASSVTPPAPAREPGHSPQ

SEQ ID NO: 44 - protein, 163 aa, Artificial Sequence
  an artificially synthesized sequence
LQDPCSNCPAGTFCDNNRNQICSPCPPNAFSSAGGQRTCDICRQCKGVFRTRKECSSTSNAECDCTPGFHCLGAGCSMCEQDCKQGQELTKKGCKDCCFGTFNDQKRGICRPWTNCSLDGKSVLVNGTKERDVVCGPSPADLSPGASSVTPPAPAREPGHSPQ

SEQ ID NO: 45 - protein, 163 aa, Artificial Sequence
  an artificially synthesized sequence
LQDPCSNCPAGTFCDNNRNQICSPCPPNSASSAGGQRTCDICRQCKGVFRTRKECSSTSNAECDCTPGFHCLGAGCSMCEQDCKQGQELTKKGCKDCCFGTFNDQKRGICRPWTNCSLDGKSVLVNGTKERDVVCGPSPADLSPGASSVTPPAPAREPGHSPQ

SEQ ID NO: 46 - protein, 163 aa, Artificial Sequence
  an artificially synthesized sequence
LQDPCSNCPAGTFCDNNRNQICSPCPPNSFASAGGQRTCDICRQCKGVFRTRKECSSTSNAECDCTPGFHCLGAGCSMCEQDCKQGQELTKKGCKDCCFGTFNDQKRGICRPWTNCSLDGKSVLVNGTKERDVVCGPSPADLSPGASSVTPPAPAREPGHSPQ

SEQ ID NO: 47 - protein, 163 aa, Artificial Sequence
  an artificially synthesized sequence
LQDPCSNCPAGTFCDNNRNQICSPCPPNSFSAAGGQRTCDICRQCKGVFRTRKECSSTSNAECDCTPGFHCLGAGCSMCEQDCKQGQELTKKGCKDCCFGTFNDQKRGICRPWTNCSLDGKSVLVNGTKERDVVCGPSPADLSPGASSVTPPAPAREPGHSPQ

SEQ ID NO: 48 - protein, 163 aa, Artificial Sequence
  an artificially synthesized sequence
LQDPCSNCPAGTFCDNNRNQICSPCPPNSFSSAAGQRTCDICRQCKGVFRTRKECSSTSNAECDCTPGFHCLGAGCSMCEQDCKQGQELTKKGCKDCCFGTFNDQKRGICRPWTNCSLDGKSVLVNGTKERDVVCGPSPADLSPGASSVTPPAPAREPGHSPQ

SEQ ID NO: 49 - protein, 163 aa, Artificial Sequence
  an artificially synthesized sequence
LQDPCSNCPAGTFCDNNRNQICSPCPPNSFSSAGAQRTCDICRQCKGVFRTRKECSSTSNAECDCTPGFHCLGAGCSMCEQDCKQGQELTKKGCKDCCFGTFNDQKRGICRPWTNCSLDGKSVLVNGTKERDVVCGPSPADLSPGASSVTPPAPAREPGHSPQ

SEQ ID NO: 50 - protein, 163 aa, Artificial Sequence
  an artificially synthesized sequence
LQDPCSNCPAGTFCDNNRNQICSPCPPNSFSSAGGARTCDICRQCKGVFRTRKECSSTSNAECDCTPGFHCLGAGCSMCEQDCKQGQELTKKGCKDCCFGTFNDQKRGICRPWTNCSLDGKSVLVNGTKERDVVCGPSPADLSPGASSVTPPAPAREPGHSPQ

SEQ ID NO: 51 - protein, 163 aa, Artificial Sequence
  an artificially synthesized sequence
LQDPCSNCPAGTFCDNNRNQICSPCPPNSFSSAGGQATCDICRQCKGVFRTRKECSSTSNAECDCTPGFHCLGAGCSMCEQDCKQGQELTKKGCKDCCFGTFNDQKRGICRPWTNCSLDGKSVLVNGTKERDVVCGPSPADLSPGASSVTPPAPAREPGHSPQ

SEQ ID NO: 52 - protein, 163 aa, Artificial Sequence
  an artificially synthesized sequence
LQDPCSNCPAGTFCDNNRNQICSPCPPNSFSSAGGQRACDICRQCKGVFRTRKECSSTSNAECDCTPGFHCLGAGCSMCEQDCKQGQELTKKGCKDCCFGTFNDQKRGICRPWTNCSLDGKSVLVNGTKERDVVCGPSPADLSPGASSVTPPAPAREPGHSPQ

SEQ ID NO: 53 - protein, 163 aa, Artificial Sequence
  an artificially synthesized sequence
LQDPCSNCPAGTFCDNNRNQICSPCPPNSFSSAGGQRTADICRQCKGVFRTRKECSSTSNAECDCTPGFHCLGAGCSMCEQDCKQGQELTKKGCKDCCFGTFNDQKRGICRPWTNCSLDGKSVLVNGTKERDVVCGPSPADLSPGASSVTPPAPAREPGHSPQ

SEQ ID NO: 54 - protein, 163 aa, Artificial Sequence
  an artificially synthesized sequence
LQDPCSNCPAGTFCDNNRNQICSPCPPNSFSSAGGQRTCAICRQCKGVFRTRKECSSTSNAECDCTPGFHCLGAGCSMCEQDCKQGQELTKKGCKDCCFGTFNDQKRGICRPWTNCSLDGKSVLVNGTKERDVVCGPSPADLSPGASSVTPPAPAREPGHSPQ

SEQ ID NO: 55 - protein, 163 aa, Artificial Sequence
  an artificially synthesized sequence
LQDPCSNCPAGTFCDNNRNQICSPCPPNSFSSAGGQRTCDACRQCKGVFRTRKECSSTSNAECDCTPGFHCLGAGCSMCEQDCKQGQELTKKGCKDCCFGTFNDQKRGICRPWTNCSLDGKSVLVNGTKERDVVCGPSPADLSPGASSVTPPAPAREPGHSPQ

SEQ ID NO: 56 - protein, 163 aa, Artificial Sequence
  an artificially synthesized sequence
LQDPCSNCPAGTFCDNNRNQICSPCPPNSFSSAGGQRTCDIARQCKGVFRTRKECSSTSNAECDCTPGFHCLGAGCSMCEQDCKQGQELTKKGCKDCCFGTFNDQKRGICRPWTNCSLDGKSVLVNGTKERDVVCGPSPADLSPGASSVTPPAPAREPGHSPQ

SEQ ID NO: 57 - protein, 163 aa, Artificial Sequence
  an artificially synthesized sequence
LQDPCSNCPAGTFCDNNRNQICSPCPPNSFSSAGGQRTCDICAQCKGVFRTRKECSSTSNAECDCTPGFHCLGAGCSMCEQDCKQGQELTKKGCKDCCFGTFNDQKRGICRPWTNCSLDGKSVLVNGTKERDVVCGPSPADLSPGASSVTPPAPAREPGHSPQ

SEQ ID NO: 58 - protein, 163 aa, Artificial Sequence
  an artificially synthesized sequence
LQDPCSNCPAGTFCDNNRNQICSPCPPNSFSSAGGQRTCDICRACKGVFRTRKECSSTSNAECDCTPGFHCLGAGCSMCEQDCKQGQELTKKGCKDCCFGTFNDQKRGICRPWTNCSLDGKSVLVNGTKERDVVCGPSPADLSPGASSVTPPAPAREPGHSPQ

SEQ ID NO: 59 - protein, 163 aa, Artificial Sequence
  an artificially synthesized sequence
LQDPCSNCPAGTFCDNNRNQICSPCPPNSFSSAGGQRTCDICRQAKGVFRTRKECSSTSNAECDCTPGFHCLGAGCSMCEQDCKQGQELTKKGCKDCCFGTFNDQKRGICRPWTNCSLDGKSVLVNGTKERDVVCGPSPADLSPGASSVTPPAPAREPGHSPQ

SEQ ID NO: 60 - protein, 163 aa, Artificial Sequence
  an artificially synthesized sequence
LQDPCSNCPAGTFCDNNRNQICSPCPPNSFSSAGGQRTCDICRQCAGVFRTRKECSSTSNAECDCTPGFHCLGAGCSMCEQDCKQGQELTKKGCKDCCFGTFNDQKRGICRPWTNCSLDGKSVLVNGTKERDVVCGPSPADLSPGASSVTPPAPAREPGHSPQ

SEQ ID NO: 61 - protein, 163 aa, Artificial Sequence
  an artificially synthesized sequence
LQDPCSNCPAGTFCDNNRNQICSPCPPNSFSSAGGQRTCDICRQCKAVFRTRKECSSTSNAECDCTPGFHCLGAGCSMCEQDCKQGQELTKKGCKDCCFGTFNDQKRGICRPWTNCSLDGKSVLVNGTKERDVVCGPSPADLSPGASSVTPPAPAREPGHSPQ

SEQ ID NO: 62 - protein, 163 aa, Artificial Sequence
  an artificially synthesized sequence
LQDPCSNCPAGTFCDNNRNQICSPCPPNSFSSAGGQRTCDICRQCKGAFRTRKECSSTSNAECDCTPGFHCLGAGCSMCEQDCKQGQELTKKGCKDCCFGTFNDQKRGICRPWTNCSLDGKSVLVNGTKERDVVCGPSPADLSPGASSVTPPAPAREPGHSPQ

SEQ ID NO: 63 - protein, 163 aa, Artificial Sequence
  an artificially synthesized sequence
LQDPCSNCPAGTFCDNNRNQICSPCPPNSFSSAGGQRTCDICRQCKGVARTRKECSSTSNAECDCTPGFHCLGAGCSMCEQDCKQGQELTKKGCKDCCFGTFNDQKRGICRPWTNCSLDGKSVLVNGTKERDVVCGPSPADLSPGASSVTPPAPAREPGHSPQ

SEQ ID NO: 64 - protein, 163 aa, Artificial Sequence
  an artificially synthesized sequence
LQDPCSNCPAGTFCDNNRNQICSPCPPNSFSSAGGQRTCDICRQCKGVFATRKECSSTSNAECDCTPGFHCLGAGCSMCEQDCKQGQELTKKGCKDCCFGTFNDQKRGICRPWTNCSLDGKSVLVNGTKERDVVCGPSPADLSPGASSVTPPAPAREPGHSPQ

SEQ ID NO: 65 - protein, 163 aa, Artificial Sequence
  an artificially synthesized sequence
LQDPCSNCPAGTFCDNNRNQICSPCPPNSFSSAGGQRTCDICRQCKGVFRARKECSSTSNAECDCTPGFHCLGAGCSMCEQDCKQGQELTKKGCKDCCFGTFNDQKRGICRPWTNCSLDGKSVLVNGTKERDVVCGPSPADLSPGASSVTPPAPAREPGHSPQ

SEQ ID NO: 66 - protein, 163 aa, Artificial Sequence
  an artificially synthesized sequence
LQDPCSNCPAGTFCDNNRNQICSPCPPNSFSSAGGQRTCDICRQCKGVFRTAKECSSTSNAECDCTPGFHCLGAGCSMCEQDCKQGQELTKKGCKDCCFGTFNDQKRGICRPWTNCSLDGKSVLVNGTKERDVVCGPSPADLSPGASSVTPPAPAREPGHSPQ

SEQ ID NO: 67 - protein, 163 aa, Artificial Sequence
  an artificially synthesized sequence
LQDPCSNCPAGTFCDNNRNQICSPCPPNSFSSAGGQRTCDICRQCKGVFRTRAECSSTSNAECDCTPGFHCLGAGCSMCEQDCKQGQELTKKGCKDCCFGTFNDQKRGICRPWTNCSLDGKSVLVNGTKERDVVCGPSPADLSPGASSVTPPAPAREPGHSPQ

SEQ ID NO: 68 - protein, 163 aa, Artificial Sequence
  an artificially synthesized sequence
LQDPCSNCPAGTFCDNNRNQICSPCPPNSFSSAGGQRTCDICRQCKGVFRTRKACSSTSNAECDCTPGFHCLGAGCSMCEQDCKQGQELTKKGCKDCCFGTFNDQKRGICRPWTNCSLDGKSVLVNGTKERDVVCGPSPADLSPGASSVTPPAPAREPGHSPQ

SEQ ID NO: 69 - protein, 163 aa, Artificial Sequence
  an artificially synthesized sequence
LQDPCSNCPAGTFCDNNRNQICSPCPPNSFSSAGGQRTCDICRQCKGVFRTRKEASSTSNAECDCTPGFHCLGAGCSMCEQDCKQGQELTKKGCKDCCFGTFNDQKRGICRPWTNCSLDGKSVLVNGTKERDVVCGPSPADLSPGASSVTPPAPAREPGHSPQ

SEQ ID NO: 70 - protein, 163 aa, Artificial Sequence
  an artificially synthesized sequence
LQDPCSNCPAGTFCDNNRNQICSPCPPNSFSSAGGQRTCDICRQCKGVFRTRKECASTSNAECDCTPGFHCLGAGCSMCEQDCKQGQELTKKGCKDCCFGTFNDQKRGICRPWTNCSLDGKSVLVNGTKERDVVCGPSPADLSPGASSVTPPAPAREPGHSPQ

SEQ ID NO: 71 - protein, 163 aa, Artificial Sequence
  an artificially synthesized sequence
LQDPCSNCPAGTFCDNNRNQICSPCPPNSFSSAGGQRTCDICRQCKGVFRTRKECSATSNAECDCTPGFHCLGAGCSMCEQDCKQGQELTKKGCKDCCFGTFNDQKRGICRPWTNCSLDGKSVLVNGTKERDVVCGPSPADLSPGASSVTPPAPAREPGHSPQ

SEQ ID NO: 72 - protein, 163 aa, Artificial Sequence
  an artificially synthesized sequence
LQDPCSNCPAGTFCDNNRNQICSPCPPNSFSSAGGQRTCDICRQCKGVFRTRKECSSASNAECDCTPGFHCLGAGCSMCEQDCKQGQELTKKGCKDCCFGTFNDQKRGICRPWTNCSLDGKSVLVNGTKERDVVCGPSPADLSPGASSVTPPAPAREPGHSPQ

SEQ ID NO: 73 - protein, 163 aa, Artificial Sequence
  an artificially synthesized sequence
LQDPCSNCPAGTFCDNNRNQICSPCPPNSFSSAGGQRTCDICRQCKGVFRTRKECSSTANAECDCTPGFHCLGAGCSMCEQDCKQGQELTKKGCKDCCFGTFNDQKRGICRPWTNCSLDGKSVLVNGTKERDVVCGPSPADLSPGASSVTPPAPAREPGHSPQ

SEQ ID NO: 74 - protein, 163 aa, Artificial Sequence
  an artificially synthesized sequence
LQDPCSNCPAGTFCDNNRNQICSPCPPNSFSSAGGQRTCDICRQCKGVFRTRKECSSTSAAECDCTPGFHCLGAGCSMCEQDCKQGQELTKKGCKDCCFGTFNDQKRGICRPWTNCSLDGKSVLVNGTKERDVVCGPSPADLSPGASSVTPPAPAREPGHSPQ

SEQ ID NO: 75 - protein, 163 aa, Artificial Sequence
  an artificially synthesized sequence
LQDPCSNCPAGTFCDNNRNQICSPCPPNSFSSAGGQRTCDICRQCKGVFRTRKECSSTSNAACDCTPGFHCLGAGCSMCEQDCKQGQELTKKGCKDCCFGTFNDQKRGICRPWTNCSLDGKSVLVNGTKERDVVCGPSPADLSPGASSVTPPAPAREPGHSPQ

SEQ ID NO: 76 - protein, 163 aa, Artificial Sequence
  an artificially synthesized sequence
LQDPCSNCPAGTFCDNNRNQICSPCPPNSFSSAGGQRTCDICRQCKGVFRTRKECSSTSNAEADCTPGFHCLGAGCSMCEQDCKQGQELTKKGCKDCCFGTFNDQKRGICRPWTNCSLDGKSVLVNGTKERDVVCGPSPADLSPGASSVTPPAPAREPGHSPQ

SEQ ID NO: 77 - protein, 163 aa, Artificial Sequence
  an artificially synthesized sequence
LQDPCSNCPAGTFCDNNRNQICSPCPPNSFSSAGGQRTCDICRQCKGVFRTRKECSSTSNAECACTPGFHCLGAGCSMCEQDCKQGQELTKKGCKDCCFGTFNDQKRGICRPWTNCSLDGKSVLVNGTKERDVVCGPSPADLSPGASSVTPPAPAREPGHSPQ

SEQ ID NO: 78 - protein, 163 aa, Artificial Sequence
  an artificially synthesized sequence
LQDPCSNCPAGTFCDNNRNQICSPCPPNSFSSAGGQRTCDICRQCKGVFRTRKECSSTSNAECDATPGFHCLGAGCSMCEQDCKQGQELTKKGCKDCCFGTFNDQKRGICRPWTNCSLDGKSVLVNGTKERDVVCGPSPADLSPGASSVTPPAPAREPGHSPQ

SEQ ID NO: 79 - protein, 163 aa, Artificial Sequence
  an artificially synthesized sequence
LQDPCSNCPAGTFCDNNRNQICSPCPPNSFSSAGGQRTCDICRQCKGVFRTRKECSSTSNAECDCAPGFHCLGAGCSMCEQDCKQGQELTKKGCKDCCFGTFNDQKRGICRPWTNCSLDGKSVLVNGTKERDVVCGPSPADLSPGASSVTPPAPAREPGHSPQ

SEQ ID NO: 80 - protein, 163 aa, Artificial Sequence
  an artificially synthesized sequence
LQDPCSNCPAGTFCDNNRNQICSPCPPNSFSSAGGQRTCDICRQCKGVFRTRKECSSTSNAECDCTAGFHCLGAGCSMCEQDCKQGQELTKKGCKDCCFGTFNDQKRGICRPWTNCSLDGKSVLVNGTKERDVVCGPSPADLSPGASSVTPPAPAREPGHSPQ

SEQ ID NO: 81 - protein, 163 aa, Artificial Sequence
  an artificially synthesized sequence
LQDPCSNCPAGTFCDNNRNQICSPCPPNSFSSAGGQRTCDICRQCKGVFRTRKECSSTSNAECDCTPAFHCLGAGCSMCEQDCKQGQELTKKGCKDCCFGTFNDQKRGICRPWTNCSLDGKSVLVNGTKERDVVCGPSPADLSPGASSVTPPAPAREPGHSPQ

SEQ ID NO: 82 - protein, 163 aa, Artificial Sequence
  an artificially synthesized sequence
LQDPCSNCPAGTFCDNNRNQICSPCPPNSFSSAGGQRTCDICRQCKGVFRTRKECSSTSNAECDCTPGAHCLGAGCSMCEQDCKQGQELTKKGCKDCCFGTFNDQKRGICRPWTNCSLDGKSVLVNGTKERDVVCGPSPADLSPGASSVTPPAPAREPGHSPQ

SEQ ID NO: 83 - protein, 163 aa, Artificial Sequence
  an artificially synthesized sequence
LQDPCSNCPAGTFCDNNRNQICSPCPPNSFSSAGGQRTCDICRQCKGVFRTRKECSSTSNAECDCTPGFACLGAGCSMCEQDCKQGQELTKKGCKDCCFGTFNDQKRGICRPWTNCSLDGKSVLVNGTKERDVVCGPSPADLSPGASSVTPPAPAREPGHSPQ

SEQ ID NO: 84 - protein, 163 aa, Artificial Sequence
  an artificially synthesized sequence
LQDPCSNCPAGTFCDNNRNQICSPCPPNSFSSAGGQRTCDICRQCKGVFRTRKECSSTSNAECDCTPGFHALGAGCSMCEQDCKQGQELTKKGCKDCCFGTFNDQKRGICRPWTNCSLDGKSVLVNGTKERDVVCGPSPADLSPGASSVTPPAPAREPGHSPQ

SEQ ID NO: 85 - protein, 163 aa, Artificial Sequence
  an artificially synthesized sequence
LQDPCSNCPAGTFCDNNRNQICSPCPPNSFSSAGGQRTCDICRQCKGVFRTRKECSSTSNAECDCTPGFHCAGAGCSMCEQDCKQGQELTKKGCKDCCFGTFNDQKRGICRPWTNCSLDGKSVLVNGTKERDVVCGPSPADLSPGASSVTPPAPAREPGHSPQ

SEQ ID NO: 86 - protein, 163 aa, Artificial Sequence
  an artificially synthesized sequence
LQDPCSNCPAGTFCDNNRNQICSPCPPNSFSSAGGQRTCDICRQCKGVFRTRKECSSTSNAECDCTPGFHCLAAGCSMCEQDCKQGQELTKKGCKDCCFGTFNDQKRGICRPWTNCSLDGKSVLVNGTKERDVVCGPSPADLSPGASSVTPPAPAREPGHSPQ

SEQ ID NO: 87 - protein, 163 aa, Artificial Sequence
  an artificially synthesized sequence
LQDPCSNCPAGTFCDNNRNQICSPCPPNSFSSAGGQRTCDICRQCKGVFRTRKECSSTSNAECDCTPGFHCLGAACSMCEQDCKQGQELTKKGCKDCCFGTFNDQKRGICRPWTNCSLDGKSVLVNGTKERDVVCGPSPADLSPGASSVTPPAPAREPGHSPQ

SEQ ID NO: 88 - protein, 163 aa, Artificial Sequence
  an artificially synthesized sequence
LQDPCSNCPAGTFCDNNRNQICSPCPPNSFSSAGGQRTCDICRQCKGVFRTRKECSSTSNAECDCTPGFHCLGAGASMCEQDCKQGQELTKKGCKDCCFGTFNDQKRGICRPWTNCSLDGKSVLVNGTKERDVVCGPSPADLSPGASSVTPPAPAREPGHSPQ

SEQ ID NO: 89 - protein, 163 aa, Artificial Sequence
  an artificially synthesized sequence
LQDPCSNCPAGTFCDNNRNQICSPCPPNSFSSAGGQRTCDICRQCKGVFRTRKECSSTSNAECDCTPGFHCLGAGCAMCEQDCKQGQELTKKGCKDCCFGTFNDQKRGICRPWTNCSLDGKSVLVNGTKERDVVCGPSPADLSPGASSVTPPAPAREPGHSPQ

SEQ ID NO: 90 - protein, 163 aa, Artificial Sequence
  an artificially synthesized sequence
LQDPCSNCPAGTFCDNNRNQICSPCPPNSFSSAGGQRTCDICRQCKGVFRTRKECSSTSNAECDCTPGFHCLGAGCSACEQDCKQGQELTKKGCKDCCFGTFNDQKRGICRPWTNCSLDGKSVLVNGTKERDVVCGPSPADLSPGASSVTPPAPAREPGHSPQ

SEQ ID NO: 91 - protein, 163 aa, Artificial Sequence
  an artificially synthesized sequence
LQDPCSNCPAGTFCDNNRNQICSPCPPNSFSSAGGQRTCDICRQCKGVFRTRKECSSTSNAECDCTPGFHCLGAGCSMAEQDCKQGQELTKKGCKDCCFGTFNDQKRGICRPWTNCSLDGKSVLVNGTKERDVVCGPSPADLSPGASSVTPPAPAREPGHSPQ

SEQ ID NO: 92 - protein, 163 aa, Artificial Sequence
  an artificially synthesized sequence
LQDPCSNCPAGTFCDNNRNQICSPCPPNSFSSAGGQRTCDICRQCKGVFRTRKECSSTSNAECDCTPGFHCLGAGCSMCAQDCKQGQELTKKGCKDCCFGTFNDQKRGICRPWTNCSLDGKSVLVNGTKERDVVCGPSPADLSPGASSVTPPAPAREPGHSPQ

SEQ ID NO: 93 - protein, 163 aa, Artificial Sequence
  an artificially synthesized sequence
LQDPCSNCPAGTFCDNNRNQICSPCPPNSFSSAGGQRTCDICRQCKGVFRTRKECSSTSNAECDCTPGFHCLGAGCSMCEADCKQGQELTKKGCKDCCFGTFNDQKRGICRPWTNCSLDGKSVLVNGTKERDVVCGPSPADLSPGASSVTPPAPAREPGHSPQ

SEQ ID NO: 94 - protein, 163 aa, Artificial Sequence
  an artificially synthesized sequence
LQDPCSNCPAGTFCDNNRNQICSPCPPNSFSSAGGQRTCDICRQCKGVFRTRKECSSTSNAECDCTPGFHCLGAGCSMCEQACKQGQELTKKGCKDCCFGTFNDQKRGICRPWTNCSLDGKSVLVNGTKERDVVCGPSPADLSPGASSVTPPAPAREPGHSPQ

SEQ ID NO: 95 - protein, 163 aa, Artificial Sequence
  an artificially synthesized sequence
LQDPCSNCPAGTFCDNNRNQICSPCPPNSFSSAGGQRTCDICRQCKGVFRTRKECSSTSNAECDCTPGFHCLGAGCSMCEQDAKQGQELTKKGCKDCCFGTFNDQKRGICRPWTNCSLDGKSVLVNGTKERDVVCGPSPADLSPGASSVTPPAPAREPGHSPQ

SEQ ID NO: 96 - protein, 163 aa, Artificial Sequence
  an artificially synthesized sequence
LQDPCSNCPAGTFCDNNRNQICSPCPPNSFSSAGGQRTCDICRQCKGVFRTRKECSSTSNAECDCTPGFHCLGAGCSMCEQDCAQGQELTKKGCKDCCFGTFNDQKRGICRPWTNCSLDGKSVLVNGTKERDVVCGPSPADLSPGASSVTPPAPAREPGHSPQ

SEQ ID NO: 97 - protein, 163 aa, Artificial Sequence
  an artificially synthesized sequence
LQDPCSNCPAGTFCDNNRNQICSPCPPNSFSSAGGQRTCDICRQCKGVFRTRKECSSTSNAECDCTPGFHCLGAGCSMCEQDCKAGQELTKKGCKDCCFGTFNDQKRGICRPWTNCSLDGKSVLVNGTKERDVVCGPSPADLSPGASSVTPPAPAREPGHSPQ

SEQ ID NO: 98 - protein, 163 aa, Artificial Sequence
  an artificially synthesized sequence
LQDPCSNCPAGTFCDNNRNQICSPCPPNSFSSAGGQRTCDICRQCKGVFRTRKECSSTSNAECDCTPGFHCLGAGCSMCEQDCKQAQELTKKGCKDCCFGTFNDQKRGICRPWTNCSLDGKSVLVNGTKERDVVCGPSPADLSPGASSVTPPAPAREPGHSPQ

SEQ ID NO: 99 - protein, 163 aa, Artificial Sequence
  an artificially synthesized sequence
LQDPCSNCPAGTFCDNNRNQICSPCPPNSFSSAGGQRTCDICRQCKGVFRTRKECSSTSNAECDCTPGFHCLGAGCSMCEQDCKQGAELTKKGCKDCCFGTFNDQKRGICRPWTNCSLDGKSVLVNGTKERDVVCGPSPADLSPGASSVTPPAPAREPGHSPQ

SEQ ID NO: 100 - protein, 163 aa, Artificial Sequence
  an artificially synthesized sequence
LQDPCSNCPAGTFCDNNRNQICSPCPPNSFSSAGGQRTCDICRQCKGVFRTRKECSSTSNAECDCTPGFHCLGAGCSMCEQDCKQGQALTKKGCKDCCFGTFNDQKRGICRPWTNCSLDGKSVLVNGTKERDVVCGPSPADLSPGASSVTPPAPAREPGHSPQ

SEQ ID NO: 101 - protein, 163 aa, Artificial Sequence
  an artificially synthesized sequence
LQDPCSNCPAGTFCDNNRNQICSPCPPNSFSSAGGQRTCDICRQCKGVFRTRKECSSTSNAECDCTPGFHCLGAGCSMCEQDCKQGQEATKKGCKDCCFGTFNDQKRGICRPWTNCSLDGKSVLVNGTKERDVVCGPSPADLSPGASSVTPPAPAREPGHSPQ

SEQ ID NO: 102 - protein, 163 aa, Artificial Sequence
  an artificially synthesized sequence
LQDPCSNCPAGTFCDNNRNQICSPCPPNSFSSAGGQRTCDICRQCKGVFRTRKECSSTSNAECDCTPGFHCLGAGCSMCEQDCKQGQELAKKGCKDCCFGTFNDQKRGICRPWTNCSLDGKSVLVNGTKERDVVCGPSPADLSPGASSVTPPAPAREPGHSPQ

SEQ ID NO: 103 - protein, 163 aa, Artificial Sequence
  an artificially synthesized sequence
LQDPCSNCPAGTFCDNNRNQICSPCPPNSFSSAGGQRTCDICRQCKGVFRTRKECSSTSNAECDCTPGFHCLGAGCSMCEQDCKQGQELTAKGCKDCCFGTFNDQKRGICRPWTNCSLDGKSVLVNGTKERDVVCGPSPADLSPGASSVTPPAPAREPGHSPQ

SEQ ID NO: 104 - protein, 163 aa, Artificial Sequence
  an artificially synthesized sequence
LQDPCSNCPAGTFCDNNRNQICSPCPPNSFSSAGGQRTCDICRQCKGVFRTRKECSSTSNAECDCTPGFHCLGAGCSMCEQDCKQGQELTKAGCKDCCFGTFNDQKRGICRPWTNCSLDGKSVLVNGTKERDVVCGPSPADLSPGASSVTPPAPAREPGHSPQ

SEQ ID NO: 105 - protein, 163 aa, Artificial Sequence
  an artificially synthesized sequence
LQDPCSNCPAGTFCDNNRNQICSPCPPNSFSSAGGQRTCDICRQCKGVFRTRKECSSTSNAECDCTPGFHCLGAGCSMCEQDCKQGQELTKKACKDCCFGTFNDQKRGICRPWTNCSLDGKSVLVNGTKERDVVCGPSPADLSPGASSVTPPAPAREPGHSPQ

SEQ ID NO: 106 - protein, 163 aa, Artificial Sequence
  an artificially synthesized sequence
LQDPCSNCPAGTFCDNNRNQICSPCPPNSFSSAGGQRTCDICRQCKGVFRTRKECSSTSNAECDCTPGFHCLGAGCSMCEQDCKQGQELTKKGAKDCCFGTFNDQKRGICRPWTNCSLDGKSVLVNGTKERDVVCGPSPADLSPGASSVTPPAPAREPGHSPQ

SEQ ID NO: 107 - protein, 163 aa, Artificial Sequence
  an artificially synthesized sequence
LQDPCSNCPAGTFCDNNRNQICSPCPPNSFSSAGGQRTCDICRQCKGVFRTRKECSSTSNAECDCTPGFHCLGAGCSMCEQDCKQGQELTKKGCADCCFGTFNDQKRGICRPWTNCSLDGKSVLVNGTKERDVVCGPSPADLSPGASSVTPPAPAREPGHSPQ

SEQ ID NO: 108 - protein, 163 aa, Artificial Sequence
  an artificially synthesized sequence
LQDPCSNCPAGTFCDNNRNQICSACPPNSFSSAGGQRTCDICRQCKGVFRTRKECSSTSNAECDCTPGFHCLGAGCSMCEQDCKQGQELTKKGCKDCCFGTFNDQKRGICRPWTNCSLDGKSVLVNGTKERDVVCGPSPADLSPGASSVTPPAPAREPGHSPQ

SEQ ID NO: 109 - protein, 163 aa, Artificial Sequence
  an artificially synthesized sequence
LQDPCSNCPAGTFCDNNRNQICAPCPPNSFSSAGGQRTCDICRQCKGVFRTRKECSSTSNAECDCTPGFHCLGAGCSMCEQDCKQGQELTKKGCKDCCFGTFNDQKRGICRPWTNCSLDGKSVLVNGTKERDVVCGPSPADLSPGASSVTPPAPAREPGHSPQ

SEQ ID NO: 110 - protein, 163 aa, Artificial Sequence
  an artificially synthesized sequence
LQDPCSNCPAGTFCDNNRNQIASPCPPNSFSSAGGQRTCDICRQCKGVFRTRKECSSTSNAECDCTPGFHCLGAGCSMCEQDCKQGQELTKKGCKDCCFGTFNDQKRGICRPWTNCSLDGKSVLVNGTKERDVVCGPSPADLSPGASSVTPPAPAREPGHSPQ

SEQ ID NO: 111 - protein, 163 aa, Artificial Sequence
  an artificially synthesized sequence
LQDPCSNCPAGTFCDNNRNQACSPCPPNSFSSAGGQRTCDICRQCKGVFRTRKECSSTSNAECDCTPGFHCLGAGCSMCEQDCKQGQELTKKGCKDCCFGTFNDQKRGICRPWTNCSLDGKSVLVNGTKERDVVCGPSPADLSPGASSVTPPAPAREPGHSPQ

SEQ ID NO: 112 - protein, 163 aa, Artificial Sequence
  an artificially synthesized sequence
LQDPCSNCPAGTFCDNNRNAICSPCPPNSFSSAGGQRTCDICRQCKGVFRTRKECSSTSNAECDCTPGFHCLGAGCSMCEQDCKQGQELTKKGCKDCCFGTFNDQKRGICRPWTNCSLDGKSVLVNGTKERDVVCGPSPADLSPGASSVTPPAPAREPGHSPQ

SEQ ID NO: 113 - protein, 163 aa, Artificial Sequence
  an artificially synthesized sequence
LQDPCSNCPAGTFCDNNRAQICSPCPPNSFSSAGGQRTCDICRQCKGVFRTRKECSSTSNAECDCTPGFHCLGAGCSMCEQDCKQGQELTKKGCKDCCFGTFNDQKRGICRPWTNCSLDGKSVLVNGTKERDVVCGPSPADLSPGASSVTPPAPAREPGHSPQ

SEQ ID NO: 114 - protein, 163 aa, Artificial Sequence
  an artificially synthesized sequence
LQDPCSNCPAGTFCDNNANQICSPCPPNSFSSAGGQRTCDICRQCKGVFRTRKECSSTSNAECDCTPGFHCLGAGCSMCEQDCKQGQELTKKGCKDCCFGTFNDQKRGICRPWTNCSLDGKSVLVNGTKERDVVCGPSPADLSPGASSVTPPAPAREPGHSPQ

SEQ ID NO: 115 - protein, 163 aa, Artificial Sequence
  an artificially synthesized sequence
LQDPCSNCPAGTFCDNARNQICSPCPPNSFSSAGGQRTCDICRQCKGVFRTRKECSSTSNAECDCTPGFHCLGAGCSMCEQDCKQGQELTKKGCKDCCFGTFNDQKRGICRPWTNCSLDGKSVLVNGTKERDVVCGPSPADLSPGASSVTPPAPAREPGHSPQ

SEQ ID NO: 116 - protein, 447 aa, Artificial Sequence
  an artificially synthesized sequence
EVQLLESGGGLVQPGGSLRLSCAASGFTFSSYAMSWVRQAPGKGLEWVSAISGSGGSTYYADSVKGRFTISRDNSKNTLYLQMNSLRAEDTAVYYCAKGWLGNFDYWGQGTLVTVSSASTKGPSVFPLAPSSKSTSGGTAALGCLVKDYFPEPVTVSWNSGALTSGVHTFPAVLQSSGLYSLSSVVTVPSSSLGTQTYICNVNHKPSNTKVDKKVEPKSCDKTHTCPPCPAPEAAGGPSVFLFPPKPKDTLMISRTPEVTCVVVDVSHEDPEVKFNWYVDGVEVHNAKTKPREEQYNSTYRVVSVLTVLHQDWLNGKEYKCKVSNKALGAPIEKTISKAKGQPREPQVCTLPPSRDELTKNQVSLSCAVKGFYPSDIAVEWESNGQPENNYKTTPPVLDSDGSFFLVSKLTVDKSRWQQGNVFSCSVMHEALHNHYTQKSLSLSPGK

SEQ ID NO: 117 - protein, 215 aa, Artificial Sequence
  an artificially synthesized sequence
EIVLTQSPGTLSLSPGERATLSCRASQSVSRSYLAWYQQKPGQAPRLLIIGASTRATGIPDRFSGSGSGTDFTLTISRLEPEDFAVYYCQQGQVIPPTFGQGTKVEIKRTVAAPSVFIFPPSDEQLKSGTASVVCLLNNFYPREAKVQWKVDNALQSGNSQESVTEQDSKDSTYSLSSTLTLSKADYEKHKVYACEVTHQGLSSPVTKSFNRGEC

SEQ ID NO: 118 - protein, 722 aa, Artificial Sequence
  an artificially synthesized sequence
REGPELSPDDPAGLLDLRQGMFAQLVAQNVLLIDGPLSWYSDPGLAGVSLTGGLSYKEDTKELVVAKAGVYYVFFQLELRRVVAGEGSGSVSLALHLQPLRSAAGAAALALTVDLPPASSEARNSAFGFQGRLLHLSAGQRLGVHLHTEARARHAWQLTQGATVLGLFRVTPEIPAGLPSPRSEGGGGSGGGGSREGPELSPDDPAGLLDLRQGMFAQLVAQNVLLIDGPLSWYSDPGLAGVSLTGGLSYKEDTKELVVAKAGVYYVFFQLELRRVVAGEGSGSVSLALHLQPLRSAAGAAALALTVDLPPASSEARNSAFGFQGRLLHLSAGQRLGVHLHTEARARHAWQLTQGATVLGLFRVTPEIPAGLPSPRSEGGGGSGGGGSRTVAAPSVFIFPPSDRKLKSGTASVVCLLNNFYPREAKVQWKVDNALQSGNSQESVTEQDSKDSTYSLSSTLTLSKADYEKHKVYACEVTHQGLSSPVTKSFNRGECDKTHTCPPCPAPEAAGGPSVFLFPPKPKDTLMISRTPEVTCVVVDVSHEDPEVKFNWYVDGVEVHNAKTKPREEQYNSTYRVVSVLTVLHQDWLNGKEYKCKVSNKALGAPIEKTISKAKGQPREPQVYTLPPCRDELTKNQVSLWCLVKGFYPSDIAVEWESNGQPENNYKTTPPVLDSDGSFFLYSKLTVDKSRWQQGNVFSCSVMHEALHNHYTQKSLSLSPGK

SEQ ID NO: 119 - protein, 297 aa, Artificial Sequence
  an artificially synthesized sequence
REGPELSPDDPAGLLDLRQGMFAQLVAQNVLLIDGPLSWYSDPGLAGVSLTGGLSYKEDTKELVVAKAGVYYVFFQLELRRVVAGEGSGSVSLALHLQPLRSAAGAAALALTVDLPPASSEARNSAFGFQGRLLHLSAGQRLGVHLHTEARARHAWQLTQGATVLGLFRVTPEIPAGLPSPRSEGGGGSGGGGSASTKGPSVFPLAPSSKSTSGGTAALGCLVEDYFPEPVTVSWNSGALTSGVHTFPAVLQSSGLYSLSSVVTVPSSSLGTQTYICNVNHKPSNTKVDEKVEPKSC

SEQ ID NO: 120 - protein, 163 aa, Artificial Sequence
  an artificially synthesized sequence
LQDPCSNCPAGTFCDNNRNQICSPCPPNSFSSAGGQRTCDICRQCKGVFRTRKECSSTSNAECDCTPGFHCLGAGCSDCEQDCKQGQELTKKGCKDCCFGTFNDQKRGICRPWTNCSLDGKSVLVNGTKERDVVCGPSPADLSPGASSVTPPAPAREPGHSPQ

SEQ ID NO: 121 - protein, 163 aa, Artificial Sequence
  an artificially synthesized sequence
LQDPCSNCPAGTFCDNNRNQICSPCPPNSFSSAGGQRTCDRCRQCKGRFRTRKECSSTSNAECDCTPGFHCLGAGCSMCEQDCKQGQELTKKGCKDCCFGTFNDQKRGICRPWTNCSLDGKSVLVNGTKERDVVCGPSPADLSPGASSVTPPAPAREPGHSPQ

SEQ ID NO: 122 - protein, 163 aa, Artificial Sequence
  an artificially synthesized sequence
LQDPCSNCPAGTFCDNNRNQICSPCPPNSFSSAGGQRTCDECRQCKGVFRTRKECSSTSNAECDCTPGFHCLGAGCSMCEQDCKQGQELTKKGCKDCCFGTFNDQKRGICRPWTNCSLDGKSVLVNGTKERDVVCGPSPADLSPGASSVTPPAPAREPGHSPQ

SEQ ID NO: 123 - protein, 163 aa, Artificial Sequence
  an artificially synthesized sequence
LQDPCSNCPAGTFCDNNRNQICSPCPPNSFSSAGGQRTCDQCRQCKGVFRTRKECSSTSNAECDCTPGFHCLGAGCSMCEQDCKQGQELTKKGCKDCCFGTFNDQKRGICRPWTNCSLDGKSVLVNGTKERDVVCGPSPADLSPGASSVTPPAPAREPGHSPQ

SEQ ID NO: 124 - protein, 163 aa, Artificial Sequence
  an artificially synthesized sequence
LQDPCSNCPAGTFCDNNRNQICSPCPPNSFSSAGGQRTCDDCRQCKGVFRTRKECSSTSNAECDCTPGFHCLGAGCSMCEQDCKQGQELTKKGCKDCCFGTFNDQKRGICRPWTNCSLDGKSVLVNGTKERDVVCGPSPADLSPGASSVTPPAPAREPGHSPQ

SEQ ID NO: 125 - protein, 163 aa, Artificial Sequence
  an artificially synthesized sequence
LQDPCSNCPAGTFCDNNRNQICSPCPPNSFSSAGGQRTCDICRQCKGEFRTRKECSSTSNAECDCTPGFHCLGAGCSMCEQDCKQGQELTKKGCKDCCFGTFNDQKRGICRPWTNCSLDGKSVLVNGTKERDVVCGPSPADLSPGASSVTPPAPAREPGHSPQ

SEQ ID NO: 126 - protein, 163 aa, Artificial Sequence
  an artificially synthesized sequence
LQDPCSNCPAGTFCDNNRNQICSPCPPNSFSSAGGQRTCDICRQCKGQFRTRKECSSTSNAECDCTPGFHCLGAGCSMCEQDCKQGQELTKKGCKDCCFGTFNDQKRGICRPWTNCSLDGKSVLVNGTKERDVVCGPSPADLSPGASSVTPPAPAREPGHSPQ

SEQ ID NO: 127 - protein, 163 aa, Artificial Sequence
  an artificially synthesized sequence
LQDPCSNCPAGTFCDNNRNQICSPCPPNSFSSAGGQRTCDICRQCKGDFRTRKECSSTSNAECDCTPGFHCLGAGCSMCEQDCKQGQELTKKGCKDCCFGTFNDQKRGICRPWTNCSLDGKSVLVNGTKERDVVCGPSPADLSPGASSVTPPAPAREPGHSPQ

SEQ ID NO: 128 - protein, 163 aa, Artificial Sequence
  an artificially synthesized sequence
LQDPCSNCPAGTFCDNNRNQICSPCPPNSFSSAGGQRTCDECRQCKGEFRTRKECSSTSNAECDCTPGFHCLGAGCSMCEQDCKQGQELTKKGCKDCCFGTFNDQKRGICRPWTNCSLDGKSVLVNGTKERDVVCGPSPADLSPGASSVTPPAPAREPGHSPQ

SEQ ID NO: 129 - protein, 163 aa, Artificial Sequence
  an artificially synthesized sequence
LQDPCSNCPAGTFCDNNRNQICSPCPPNSFSSAGGQRTCDECRQCKGQFRTRKECSSTSNAECDCTPGFHCLGAGCSMCEQDCKQGQELTKKGCKDCCFGTFNDQKRGICRPWTNCSLDGKSVLVNGTKERDVVCGPSPADLSPGASSVTPPAPAREPGHSPQ

SEQ ID NO: 130 - protein, 163 aa, Artificial Sequence
  an artificially synthesized sequence
LQDPCSNCPAGTFCDNNRNQICSPCPPNSFSSAGGQRTCDECRQCKGDFRTRKECSSTSNAECDCTPGFHCLGAGCSMCEQDCKQGQELTKKGCKDCCFGTFNDQKRGICRPWTNCSLDGKSVLVNGTKERDVVCGPSPADLSPGASSVTPPAPAREPGHSPQ

SEQ ID NO: 131 - protein, 163 aa, Artificial Sequence
  an artificially synthesized sequence
LQDPCSNCPAGTFCDNNRNQICSPCPPNSFSSAGGQRTCDQCRQCKGEFRTRKECSSTSNAECDCTPGFHCLGAGCSMCEQDCKQGQELTKKGCKDCCFGTFNDQKRGICRPWTNCSLDGKSVLVNGTKERDVVCGPSPADLSPGASSVTPPAPAREPGHSPQ

SEQ ID NO: 132 - protein, 163 aa, Artificial Sequence
  an artificially synthesized sequence
LQDPCSNCPAGTFCDNNRNQICSPCPPNSFSSAGGQRTCDQCRQCKGQFRTRKECSSTSNAECDCTPGFHCLGAGCSMCEQDCKQGQELTKKGCKDCCFGTFNDQKRGICRPWTNCSLDGKSVLVNGTKERDVVCGPSPADLSPGASSVTPPAPAREPGHSPQ

SEQ ID NO: 133 - protein, 163 aa, Artificial Sequence
  an artificially synthesized sequence
LQDPCSNCPAGTFCDNNRNQICSPCPPNSFSSAGGQRTCDQCRQCKGDFRTRKECSSTSNAECDCTPGFHCLGAGCSMCEQDCKQGQELTKKGCKDCCFGTFNDQKRGICRPWTNCSLDGKSVLVNGTKERDVVCGPSPADLSPGASSVTPPAPAREPGHSPQ

SEQ ID NO: 134 - protein, 163 aa, Artificial Sequence
  an artificially synthesized sequence
LQDPCSNCPAGTFCDNNRNQICSPCPPNSFSSAGGQRTCDDCRQCKGEFRTRKECSSTSNAECDCTPGFHCLGAGCSMCEQDCKQGQELTKKGCKDCCFGTFNDQKRGICRPWTNCSLDGKSVLVNGTKERDVVCGPSPADLSPGASSVTPPAPAREPGHSPQ

SEQ ID NO: 135 - protein, 163 aa, Artificial Sequence
  an artificially synthesized sequence
LQDPCSNCPAGTFCDNNRNQICSPCPPNSFSSAGGQRTCDDCRQCKGQFRTRKECSSTSNAECDCTPGFHCLGAGCSMCEQDCKQGQELTKKGCKDCCFGTFNDQKRGICRPWTNCSLDGKSVLVNGTKERDVVCGPSPADLSPGASSVTPPAPAREPGHSPQ

SEQ ID NO: 136 - protein, 163 aa, Artificial Sequence
  an artificially synthesized sequence
LQDPCSNCPAGTFCDNNRNQICSPCPPNSFSSAGGQRTCDDCRQCKGDFRTRKECSSTSNAECDCTPGFHCLGAGCSMCEQDCKQGQELTKKGCKDCCFGTFNDQKRGICRPWTNCSLDGKSVLVNGTKERDVVCGPSPADLSPGASSVTPPAPAREPGHSPQ

SEQ ID NO: 137 - protein, 163 aa, Artificial Sequence; identical to SEQ ID NO: 36
  an artificially synthesized sequence

SEQ ID NO: 138 - protein, 157 aa, Artificial Sequence
  an artificially synthesized sequence
LQDPCSNCPAGTFCDNNRNQICSPCPPNSFSSAGGQRTCDICRQCKGVFRTRKECSSTSNAECDCTPGFHCLGAGCSMCEQDCKQGQELTKKGCKDCCFGTFNDQKRGICRPWTNCSLDGKSVLVNGTKERDVVCGPSPADLSPGASSVTPPAPARE

SEQ ID NO: 139 - protein, 138 aa, Artificial Sequence
  an artificially synthesized sequence
SLQDPCSNCPAGTFCDNNRNQICSPCPPNSFSSAGGQRTCDICRQCKGVFRTRKECSSTSNAECDCTPGFHCLGAGCSMCEQDCKQGQELTKKGCKDCCFGTFNDQKRGICRPWTNCSLDGKSVLVNGTKERDVVCGP

SEQ ID NO: 140 - protein, 138 aa, Artificial Sequence
  an artificially synthesized sequence
QDPCSNCPAGTFCDNNRNQICSPCPPNSFSSAGGQRTCDICRQCKGVFRTRKECSSTSNAECDCTPGFHCLGAGCSMCEQDCKQGQELTKKGCKDCCFGTFNDQKRGICRPWTNCSLDGKSVLVNGTKERDVVCGPSP